European Patent Specification EP 4 081 657 B1, published October 29, 2025. Title: NANOPARTICLE WITH SINGLE SITE FOR TEMPLATE POLYNUCLEOTIDE ATTACHMENT. Applicant: ILLUMINA, INC. ILLUMINA CAMBRIDGE LIMITED ILLUMINA SINGAPORE PTE. LTD. The sequence listing filed with the application follows.

SEQUENCE LISTING (8 sequences)

SEQ ID NO: 1 - protein, 13 aa, Artificial Sequence
  Laboratory-synthesized sequence
AHIVMVDAYKPTK

SEQ ID NO: 2 - protein, 134 aa, Artificial Sequence
  Laboratory-synthesized sequence
MKGSSHHHHHHVDIPTTENLYFQGAMVDTLSGLSSEQGQSGDMTIEEDSATHIKFSKRDEDGKELAGATMELRDSSGKTISTWISDGQVKDFYLYPGKYTFVETAAPDGYEVATAITFTVNEQGQVTVNGKATK

SEQ ID NO: 3 - protein, 15 aa, Artificial Sequence
  Laboratory-synthesized sequence
GLNDIFEAQKIEWHE

SEQ ID NO: 4 - protein, 11 aa, Artificial Sequence
  Laboratory-synthesized sequence
DSLEFIASKLA

SEQ ID NO: 5 - protein, 22 aa, Artificial Sequence
  Laboratory-synthesized sequence
DEVLVEIETDKAVLEVPGGEEE

SEQ ID NO: 6 - protein, 13 aa, Artificial Sequence
  Laboratory-synthesized sequence
GFEIDKVWYDLDA

SEQ ID NO: 7 - DNA, 29 bp, Artificial Sequence
  Laboratory-synthesized sequence
aatgatacggcgaccaccgagatctacac

SEQ ID NO: 8 - DNA, 24 bp, Artificial Sequence
  Laboratory-synthesized sequence
caagcagaagacggcatacgagat